European Patent Application EP 4 725 508 A1, published April 15, 2026. Title: 一种自带游离载荷回收单元的配体药物偶联物. Applicant: 荣昌生物制药（烟台）股份有限公司. Application CN. The sequence listing filed with the application follows.

SEQUENCE LISTING (164 sequences)

SEQ ID NO: 1 - protein, 120 aa, synthetic construct
EVQLQESGPGLVKSFQTVSLTCTVTGYSITNANHWWNWFRQVSGSKLEWIGYISSSGTTDINPSLKSRFSITRDTSKNQLFLQLNAVTTEDIATYFCVRTYYDGTYEENWGPGTTLTVSS

SEQ ID NO: 2 - protein, 10 aa, synthetic construct
GYSITNANHW

SEQ ID NO: 3 - protein, 7 aa, synthetic construct
ISSSGTT

SEQ ID NO: 4 - protein, 12 aa, synthetic construct
VRTYYDGTYEEN

SEQ ID NO: 5 - protein, 107 aa, synthetic construct
DIVMTQTPKFLPVSAGDRVTMTCKASQSVGNNVAWYQQKPGQSPKLLIYYASNRYTGVPDRFTGSGSGTDFTFTISSVQVEDLAVYFCQQHYNSPWTFAGGTKLEIK

SEQ ID NO: 6 - protein, 6 aa, synthetic construct
QSVGNN

SEQ ID NO: 7 - protein, 13 aa, synthetic construct
QQHYNSPWTFAGG

SEQ ID NO: 8 - protein, 120 aa, synthetic construct
EVQLQESGPGLVKPSQTVSLTCTVTGNSITNTNNWWNWIRQVSGSKLEWIGYISSSGSTDSNPSLKSRISITRDTSRNQLFLQLKSVTPEDVATYYCVRTYYDGSYEENWGQGTTLTVSS

SEQ ID NO: 9 - protein, 10 aa, synthetic construct
GNSITNTNNW

SEQ ID NO: 10 - protein, 7 aa, synthetic construct
ISSSGST

SEQ ID NO: 11 - protein, 12 aa, synthetic construct
VRTYYDGSYEEN

SEQ ID NO: 12 - protein, 107 aa, synthetic construct
DIVMTQTPKFLPVSARDRATMTCKASQSVGNNVAWYQQKPGQSPKLLIYFASKRYTGVPDRFTGRGSGTDFTFTISSVQVEDLAVYFCQQHYISPWTFGGGTKLELK

SEQ ID NO: 13 - protein, 9 aa, synthetic construct
QQHYISPWT

SEQ ID NO: 14 - protein, 120 aa, synthetic construct
QVQLQESGPGLVKPSQTLSLTCTVSGYSITNANHWWSWIRQPPGKGLEWIGYISSSGTTYYNPSLKSRVTISVDTSKNQFSLKLSSVTAADTAVYYCVRTYYDGTYEENWGQGTTVTVSS

SEQ ID NO: 15 - protein, 107 aa, synthetic construct
DIQMTQSPSSLSASVGDRVTITCQASQSVGNNLNWYQQKPGKAPKLLIYYASNLETGVPSRFSGSGSGTDFTFTISSLQPEDIATYYCQQHYNSPWTFGGGTKVEIK

SEQ ID NO: 16 - protein, 9 aa, synthetic construct
QQHYNSPWT

SEQ ID NO: 17 - protein, 120 aa, synthetic construct
QVQLQESGPGLVKPSQTLSLTCTVSGYSITNANHWWNWFRQPPGKGLEWIGYISSSGTTDINPSLKSRVTISRDTSKNQLSLKLSSVTAADTAVYYCVRTYYDGTYEENWGQGTTVTVSS

SEQ ID NO: 18 - protein, 107 aa, synthetic construct
DIQMTQSPSSLSASVGDRVTITCQASQSVGNNVAWYQQKPGKAPKLLIYYASNLYTGVPSRFSGSGSGTDFTFTISSLQPEDIATYFCQQHYNSPWTFAGGTKVEIK

SEQ ID NO: 19 - protein, 120 aa, synthetic construct
QVQLQESGPGLVKPSQTLSLTCTVSGYSITNANHWWNWFRQPPGKGLEWIGYISSSGTTDINPSLKSRVTISRDTSKNQLSLKLSSVTAADTAVYYCVRTYYDSTYEENWGQGTTVTVSS

SEQ ID NO: 20 - protein, 12 aa, synthetic construct
VRTYYDSTYEEN

SEQ ID NO: 21 - protein, 121 aa, synthetic construct
EVQMQQSGAELVKPGASVKLSCKTSGFTFSSSYISWLKQKPGQSLEWIAWIYAGTGNTNYNQKFAGRAQLTVDTSSSTAYMQFSGLTTEDSAIYYCSRDGYDGRSYDLDYWGQGTSVTVSS

SEQ ID NO: 22 - protein, 8 aa, synthetic construct
GFTFSSSY

SEQ ID NO: 23 - protein, 8 aa, synthetic construct
IYAGTGNT

SEQ ID NO: 24 - protein, 14 aa, synthetic construct
SRDGYDGRSYDLDY

SEQ ID NO: 25 - protein, 107 aa, synthetic construct
DVVLTQSHKFMSTSVGDRVSITCKASQDVGTSVAWYQQKPGQSPKLLIYWASTRHTGVPDRFTGSGSGTDFTLTIGNVQSEDLADYFCQQFSTYPLTFGGGTKLEIK

SEQ ID NO: 26 - protein, 6 aa, synthetic construct
QDVGTS

SEQ ID NO: 27 - protein, 9 aa, synthetic construct
QQFSTYPLT

SEQ ID NO: 28 - protein, 120 aa, synthetic construct
EVQLQQSGPELVKPGASVKMSCKASGYTFTSYVMHWVKQKPGQGLEWIGYIIHYNDVTKYNENFRGKATLTSDKSSSTAYMEVSSLTSEDSAVYYCTRSPYYYDGSFDYWGQGTTLTVSS

SEQ ID NO: 29 - protein, 8 aa, synthetic construct
GYTFTSYV

SEQ ID NO: 30 - protein, 8 aa, synthetic construct
IIHYNDVT

SEQ ID NO: 31 - protein, 13 aa, synthetic construct
TRSPYYYDGSFDY

SEQ ID NO: 32 - protein, 112 aa, synthetic construct
DVVMTQTPLSLPVSLGDQASISCRSSQSIVHSNGNTYLEWFLQKPGQSPKLLIYKVSNRFSGVPDRFSGSGSGTDFTLKISRVEAEDLGVYYCFQGSHAPYTFGGGTKLEIK

SEQ ID NO: 33 - protein, 11 aa, synthetic construct
QSIVHSNGNTY

SEQ ID NO: 34 - protein, 9 aa, synthetic construct
FQGSHAPYT

SEQ ID NO: 35 - protein, 120 aa, synthetic construct
QVQLQQSGPELVKPGASVKMSCKASGYTFTSYVMHWVKQKPGQGLEWIGYIIHYNDGTKYNEKFRGKATLTSDKSSSTAYMELSSLTSEDSAVYYCARSPYYSDGSFDYWGQGTTLTVSS

SEQ ID NO: 36 - protein, 8 aa, synthetic construct
IIHYNDGT

SEQ ID NO: 37 - protein, 13 aa, synthetic construct
ARSPYYSDGSFDY

SEQ ID NO: 38 - protein, 112 aa, synthetic construct
DILMTQTPLSLPVSLGDQASISCRSSQSIVHSNGNTYLEWFLQKPGQSPKLLIYKLSNRFSGVPDRFSGSGSGTDFTLKISRVEAEDLGVYYCFQGSHAPYTFGGGTKLEIK

SEQ ID NO: 39 - protein, 120 aa, synthetic construct
EVQLVESGGGLVKPGGSLKLSCAASGFTFSAYYMHWIRQTPEERLEWVATISDGGSNTYYPDSVKGRFIISRDNAKNILYLQMSSLKSEDTAMYYCARDGGWLLYYFDYWGQGTTLTVSS

SEQ ID NO: 40 - protein, 8 aa, synthetic construct
GFTFSAYY

SEQ ID NO: 41 - protein, 8 aa, synthetic construct
ISDGGSNT

SEQ ID NO: 42 - protein, 13 aa, synthetic construct
ARDGGWLLYYFDY

SEQ ID NO: 43 - protein, 112 aa, synthetic construct
DVVMTQTPLSLPVSLGDQASISCRSSQAIVQSNGETYLEWYLQKSGQSPKLLIYKVSNRFTGVPDRFSGSGSGTDFTLKISRVEAEDLGVYYCFQGSHVPWTFGGGTKLEIK

SEQ ID NO: 44 - protein, 11 aa, synthetic construct
QAIVQSNGETY

SEQ ID NO: 45 - protein, 9 aa, synthetic construct
FQGSHVPWT

SEQ ID NO: 46 - protein, 120 aa, synthetic construct
EVQLVESGGGLVKPGGSLKLSCAASGFIFSDHYMYWVRQTPEKRLEWVAVISDGGTYTNYPDSVKGRFTISRDNAKNTLYLHIHSLKSEDTAMYYCARDGGWLLYYFDYWGQGTTLTVSS

SEQ ID NO: 47 - protein, 8 aa, synthetic construct
GFIFSDHY

SEQ ID NO: 48 - protein, 8 aa, synthetic construct
ISDGGTYT

SEQ ID NO: 49 - protein, 112 aa, synthetic construct
DVVLTQTPLSLPVSLGDQASISCRSSQNIVQSDGNTYLEWYLQKPGQSPKLLIYKVSNRFSGVPDRFSGSGSGTDFTLKISRVEAEDLGVYYCFQGSHLPWTFGGGTKLEIK

SEQ ID NO: 50 - protein, 11 aa, synthetic construct
QNIVQSDGNTY

SEQ ID NO: 51 - protein, 9 aa, synthetic construct
FQGSHLPWT

SEQ ID NO: 52 - protein, 114 aa, synthetic construct
EVQLVESGGGLVKPGGSLKLSCAASGFTFSDNYMYWVRQTPEKRLEWVATISAGGSYTYYPDSVKGRFTISRDNAKNNLYLQMSSLKSEDTAMYYCAGTAMDYWGQGTSVTVSS

SEQ ID NO: 53 - protein, 8 aa, synthetic construct
GFTFSDNY

SEQ ID NO: 54 - protein, 8 aa, synthetic construct
ISAGGSYT

SEQ ID NO: 55 - protein, 7 aa, synthetic construct
AGTAMDY

SEQ ID NO: 56 - protein, 106 aa, synthetic construct
DIVLTQSPAIMSASPGEKVTMTCSASSSVSYMHWYQQKSGTSPKRWIYDTSKLASGVPARFSGSGSGTSYSLTISSLEAEDAATYYCLQWKSYPPTFGAGTKLEIK

SEQ ID NO: 57 - protein, 5 aa, synthetic construct
SSVSY

SEQ ID NO: 58 - protein, 9 aa, synthetic construct
LQWKSYPPT

SEQ ID NO: 59 - protein, 114 aa, synthetic construct
EVQLVESGGGLVKPGGSLKLSCAASGFTFSDNYMYWVRQTPEKRLEWVATISAGGSYTYYPDSVKGRFTISRDNAMNNLYLQMSSLKSEDTAMYYCAGTAMDYWGQGTSVTVSS

SEQ ID NO: 60 - protein, 106 aa, synthetic construct; identical to SEQ ID NO: 56

SEQ ID NO: 61 - protein, 118 aa, synthetic construct
EVQLQESGGGLVQPGGSMKLSCVASGFTFINYWMNWVRQSPERGLEWVAQISLISDDYATHYAESVKGRFTISRDDSKSSLYLQMNNLRAEDTGIYYCTEAGYFFDYWGQGTTLTVSS

SEQ ID NO: 62 - protein, 8 aa, synthetic construct
GFTFINYW

SEQ ID NO: 63 - protein, 10 aa, synthetic construct
ISLISDDYAT

SEQ ID NO: 64 - protein, 9 aa, synthetic construct
TEAGYFFDY

SEQ ID NO: 65 - protein, 107 aa, synthetic construct
DVVMTQSQQFMSTSVGDRVSVTCKASQNVGTNVAWYQQRPGQSPKALIYSASYRYSGVPDRFTGSGSGTDFTLTISNVQSEDLAEYFCQQYNSYPLTFGAGTKLELK

SEQ ID NO: 66 - protein, 6 aa, synthetic construct
QNVGTN

SEQ ID NO: 67 - protein, 9 aa, synthetic construct
QQYNSYPLT

SEQ ID NO: 68 - protein, 116 aa, synthetic construct
EVQLQESGGGLVQPGGSMKLSCVASGFTLSNYWMNWVRQSPEKGLEWVAQIRPKSYNYATHYAESVKGRFTISRDGSKSSVYLEMSNLRAEDTGIYYCTGFPFDYWGQGTTLTVSS

SEQ ID NO: 69 - protein, 8 aa, synthetic construct
GFTLSNYW

SEQ ID NO: 70 - protein, 10 aa, synthetic construct
IRPKSYNYAT

SEQ ID NO: 71 - protein, 7 aa, synthetic construct
TGFPFDY

SEQ ID NO: 72 - protein, 107 aa, synthetic construct
DIVMTQSHKFMSTSVGDRVSITCKASQDVGTAVAWYQQKPGQSPKLLIYWASTRHTGVPDRFTGSGSWTDFTLTINNVQSEDLADYFCQQYSSYPLTFGAGTKLEIK

SEQ ID NO: 73 - protein, 6 aa, synthetic construct
QDVGTA

SEQ ID NO: 74 - protein, 9 aa, synthetic construct
QQYSSYPLT

SEQ ID NO: 75 - protein, 120 aa, synthetic construct
DVQLQESGPGLVKPSQTVSLTCTVTGISITNGNHWWNWIRQLSGNKLEWIGYIRPSGSTDSNPSLKSRISITRDTSKNQVFLQLNSVTPEDVATYYCARGGLEDGKYYYAMDYWGQGTSL

SEQ ID NO: 76 - protein, 10 aa, synthetic construct
GISITNGNHW

SEQ ID NO: 77 - protein, 7 aa, synthetic construct
IRPSGST

SEQ ID NO: 78 - protein, 16 aa, synthetic construct
ARGGLEDGKYYYAMDY

SEQ ID NO: 79 - protein, 111 aa, synthetic construct
DIVLTQSPPSLAVSLGQSVTISCRASENVEYFGTSLMQWYQQKPGQPPKLLIYGASSVESGVPARFSGSGSGTDFSLKIHPVEEDDIAMYFCQQSRKVPSTFGSGTKLEIK

SEQ ID NO: 80 - protein, 10 aa, synthetic construct
ENVEYFGTSL

SEQ ID NO: 81 - protein, 9 aa, synthetic construct
QQSRKVPST

SEQ ID NO: 82 - protein, 122 aa, synthetic construct
DVQLQESGGGLVQPGGSMKLSCIASGFTFTNYWMNWVRQSPEKGLEWVAQIRLMSNNCATHYAESVKGRFTISRDASKSFFYLQMNNLRAEDTGIYYCTYYDYDYYYSMDYWGQGTSVTVSS

SEQ ID NO: 83 - protein, 8 aa, synthetic construct
GFTFTNYW

SEQ ID NO: 84 - protein, 10 aa, synthetic construct
IRLMSNNCAT

SEQ ID NO: 85 - protein, 13 aa, synthetic construct
TYYDYDYYYSMDY

SEQ ID NO: 86 - protein, 107 aa, synthetic construct
DVVMTQSQKFMSTSVGDRVSVTCKASQNVATNVAWYQQKPGQSPKALFYSASYRYSGVPDRFTGSGSGTDFTLTISNVQSEDLAEYFCQQYNSYPLTFGAGTKLEIK

SEQ ID NO: 87 - protein, 6 aa, synthetic construct
QNVATN

SEQ ID NO: 88 - protein, 116 aa, synthetic construct
EVQLQQSGPELVKPGASVKMSCKASGHTFTSYVMNWVKQKPGLGLDWIGYINPYNGGIKYNEKFKGKATLTSDKSSRTAYMELSSLTSEDSAVYYCYYYGNSYGYWGQGTTLTVSS

SEQ ID NO: 89 - protein, 8 aa, synthetic construct
GHTFTSYV

SEQ ID NO: 90 - protein, 8 aa, synthetic construct
INPYNGGI

SEQ ID NO: 91 - protein, 9 aa, synthetic construct
YYYGNSYGY

SEQ ID NO: 92 - protein, 107 aa, synthetic construct
DILMTQSPSSMSVSLGDTVSITCHASQGINSNIGWLQQKPGKSFKGLIYHGTNLEDGVPSRFSGGGSGADYSLTISSLESEDFADYYCIQYAQFPFTFGSGTKLEIK

SEQ ID NO: 93 - protein, 6 aa, synthetic construct
QGINSN

SEQ ID NO: 94 - protein, 9 aa, synthetic construct
IQYAQFPFT

SEQ ID NO: 95 - protein, 124 aa, synthetic construct
QVQLQESGPGLVKPSQTLSLTCTVSGISITNGNHWWSWIRQPPGKGLEWIGYIRPSGSTYYNPSLKSRVTISVDTSKNQFSLKLSSVTAADTAVYYCARGGLEDGKYYYAMDYWGQGTTVTVSS

SEQ ID NO: 96 - protein, 111 aa, synthetic construct
DIVMTQSPDSLAVSLGERATINCKSSENVEYFGTSLLAWYQQKPGQPPKLLIYGASTRESGVPDRFSGSGSGTDFTLTISSLQAEDVAVYYCQQSRKVPSTFGQGTKLEIK

SEQ ID NO: 97 - protein, 124 aa, synthetic construct
QVQLQESGPGLVKPSQTLSLTCTVSGISITNGNHWWNWIRQPPGKGLEWIGYIRPSGSTYSNPSLKSRVTISRDTSKNQVSLKLSSVTAADTAVYYCARGGLEDGKYYYAMDYWGQGTTVTVSS

SEQ ID NO: 98 - protein, 124 aa, synthetic construct
QVQLQESGPGLVKPSQTLSLTCTVSGISITNANHWWNWIRQPPGKGLEWIGYIRPSGSTYSNPSLKSRVTISRDTSKNQVSLKLSSVTAADTAVYYCARGGLEEGKYYYAMDYWGQGTTVTVSS

SEQ ID NO: 99 - protein, 10 aa, synthetic construct
GISITNANHW

SEQ ID NO: 100 - protein, 16 aa, synthetic construct
ARGGLEEGKYYYAMDY

SEQ ID NO: 101 - protein, 351 aa, synthetic construct
QVQLQESGGGLVQPGGSLRLSCAASGFTFSIYYMGWVRQAPGKGPEWVSAINTGGGSTWYADSVKGRFTISRDNAKNTLYLQMNSLKPEDTALYYCARVLDPSTWEYDTWGQGTQVTVSSEPKSCDKTHTCPPCPAPELLGGPSVFLFPPKPKDTLMISRTPEVTCVVVDVSHEDPEVKFNWYVDGVEVHNAKTKPREEQYNSTYRVVSVLTVLHQDWLNGKEYKCKVSNKALPAPIEKTISKAKGQPREPQVYTLPPSRDELTKNQVSLTCLVKGFYPSDIAVEWESNGQPENNYKTTPPVLDSDGSFFLYSKLTVDKSRWQQGNVFSCSVMHEALHNHYTQKSLSLSPG

SEQ ID NO: 102 - protein, 120 aa, synthetic construct
QVQLQESGGGLVQPGGSLRLSCAASGFTFSIYYMGWVRQAPGKGPEWVSAINTGGGSTWYADSVKGRFTISRDNAKNTLYLQMNSLKPEDTALYYCARVLDPSTWEYDTWGQGTQVTVSS

SEQ ID NO: 103 - protein, 8 aa, synthetic construct
GFTFSIYY

SEQ ID NO: 104 - protein, 8 aa, synthetic construct
INTGGGST

SEQ ID NO: 105 - protein, 13 aa, synthetic construct
ARVLDPSTWEYDT

SEQ ID NO: 106 - protein, 15 aa, synthetic construct
ACDESHGVPHTSGMC

SEQ ID NO: 107 - protein, 15 aa, synthetic construct
ACLPNSLGPSAMSSC

SEQ ID NO: 108 - protein, 15 aa, synthetic construct
ACLVLKLSTGIKSEC

SEQ ID NO: 109 - protein, 15 aa, synthetic construct
ACRLTGPDWLHTQRC

SEQ ID NO: 110 - protein, 11 aa, synthetic construct
ACTPALRSLAC

SEQ ID NO: 111 - protein, 11 aa, synthetic construct
ACLRNSPRKQC

SEQ ID NO: 112 - protein, 15 aa, synthetic construct
ACHWNAKADYGSFVC

SEQ ID NO: 113 - protein, 15 aa, synthetic construct
ACTGCSRTHSPRSRC

SEQ ID NO: 114 - protein, 11 aa, synthetic construct
ACVLSPHPQAC

SEQ ID NO: 115 - protein, 11 aa, synthetic construct
ACDSLGGSPVC

SEQ ID NO: 116 - protein, 245 aa, synthetic construct
ACDESHGVPHTSGMCGGGSDKTHTCPPCPAPELLGGPSVFLFPPKPKDTLMISRTPEVTCVVVDVSHEDPEVKFNWYVDGVEVHNAKTKPREEQYNSTYRVVSVLTVLHQDWLNGKEYKCKVSNKALPAPIEKTISKAKGQPREPQVYTLPPSREEMTKNQVSLTCLVKGFYPSDIAVEWESNGQPENNYKTTPPVLDSDGSFFLYSKLTVDKSRWQQGNVFSCSVMHEALHNHYTQKSLSLSPG

SEQ ID NO: 117 - protein, 363 aa, synthetic construct
ACDESHGVPHTSGMCGGGSEVQLVESGGGLVQPGGSLRLSCAVSGFPLSSYGMSWARQAPGEERELVAHIGTTGGSTNYADSVKGRFTISRDNAKNSVYLQMNSLRAEDTAVYYCRARRQMPSNEYWGQGTTVTVSSDKTHTCPPCPAPELLGGPSVFLFPPKPKDTLMISRTPEVTCVVVDVSHEDPEVKFNWYVDGVEVHNAKTKPREEQYNSTYRVVSVLTVLHQDWLNGKEYKCKVSNKALPAPIEKTISKAKGQPREPQVYTLPPSREEMTKNQVSLTCLVKGFYPSDIAVEWESNGQPENNYKTTPPVLDSDGSFFLYSKLTVDKSRWQQGNVFSCSVMHEALHNHYTQKSLSLSPG

SEQ ID NO: 118 - protein, 15 aa, synthetic construct
VALTWYYPIYLFATR

SEQ ID NO: 119 - protein, 15 aa, synthetic construct
ILTTVNVVPNTIHVR

SEQ ID NO: 120 - protein, 11 aa, synthetic construct
ACLACWTSRSC

SEQ ID NO: 121 - protein, 11 aa, synthetic construct
ACLSPWLFFWC

SEQ ID NO: 122 - protein, 15 aa, synthetic construct
ACYPFGNPRGVRPSC

SEQ ID NO: 123 - protein, 15 aa, synthetic construct
ACWTLWLPLLPLGSC

SEQ ID NO: 124 - protein, 15 aa, synthetic construct
ACGSLSWRNCGSYRC

SEQ ID NO: 125 - protein, 15 aa, synthetic construct
ACSQCVLLPPPQSVC

SEQ ID NO: 126 - protein, 15 aa, synthetic construct
AHNVEILPPFDYTLS

SEQ ID NO: 127 - protein, 15 aa, synthetic construct
LTVAMITTSRITTSN

SEQ ID NO: 128 - protein, 15 aa, synthetic construct
APPTFPVSTSVVISR

SEQ ID NO: 129 - protein, 7 aa, synthetic construct
YYVAWRW

SEQ ID NO: 130 - protein, 239 aa, synthetic construct
DKTHTCPPCPAPELLGGPSVFLFPPKPKDTLMISRTPEVTCVVVDVSHEDPEVKFNWYVDGVEVHNAKTKPREEQYNSTYRVVSVLTVLHQDWLNGKEYKCKVSNKALPAPIEKTISKAKGQPREPQVYTLPPSREEMTKNQVSLTCLVKGFYPSDIAVEWESNGQPENNYKTTPPVLDSDGSFFLYSKLTVDKSRWQQGNVFSCSVMHEALHNHYTQKSLSLSPGGSGGGSYYVAWRW

SEQ ID NO: 131 - DNA, 66 bp, synthetic construct
  source 1..66: mol_type = other DNA
cagcaccgtcaactgaatgaaatgcgtgaaagttcgaaaatagttctcgtgatgcgatggagatgt

SEQ ID NO: 132 - DNA, 66 bp, synthetic construct
  source 1..66: mol_type = other DNA
cagcaccgtcaactgaatcggggcacgcaattcgtagtgttaagttgtgtgatgcgatggagatgt

SEQ ID NO: 133 - DNA, 66 bp, synthetic construct
  source 1..66: mol_type = other DNA
cagcaccgtcaactgaatctacgcgtgatgcatattggtcgagcgggggtgatgcgatggagatgt

SEQ ID NO: 134 - DNA, 66 bp, synthetic construct
  source 1..66: mol_type = other DNA
cagcaccgtcaactgaatgaaaagcgcaaatctggctaacataggctcgtgatgcgatggagatgt

SEQ ID NO: 135 - DNA, 66 bp, synthetic construct
  source 1..66: mol_type = other DNA
cagcaccgtcaactgaatgatccagaaaacggcgaccgtctcagcgtagtgatgcgatggagatgt

SEQ ID NO: 136 - DNA, 66 bp, synthetic construct
  source 1..66: mol_type = other DNA
cagcaccgtcaactgaatagattcaaggtcttgccgggatatcgccatgtgatgcgatggagatgt

SEQ ID NO: 137 - DNA, 110 bp, synthetic construct
  source 1..110: mol_type = other DNA
cctgccacgctccgcaagcttagtcatagtactgcagcgattcttgatcgtaatactagctaactcttggcactagaagagattgagtcctaagcttgcacccgcatcgt

SEQ ID NO: 138 - DNA, 110 bp, synthetic construct
  source 1..110: mol_type = other DNA
cctgccacgctccgcaagctttgaacggattctgcagcgattcttgatcgttacttgggcattatcgtcatcagctttcatgagtaagggtaagcttgcacccgcatcgt

SEQ ID NO: 139 - DNA, 109 bp, synthetic construct
  source 1..109: mol_type = other DNA
cctgccacgctccgcaagcttctattgacttctgcaggattcttgatcgcaaacattgtcagatgcgaggttgacagctgtagttacactaagcttgcacccgcatcgt

SEQ ID NO: 140 - DNA, 110 bp, synthetic construct
  source 1..110: mol_type = other DNA
cctgccacgctccgcaagcttcctatcatgcctgcagcgattcttgatcggattagtgtttgctacctgtttctagcagtccgtagctcataagcttgcacccgcatcgt

SEQ ID NO: 141 - DNA, 110 bp, synthetic construct
  source 1..110: mol_type = other DNA
cctgccacgctccgcaagcttgttatacgccctgcagcgattcttgatcgttcgtctccgatcccagccttactaccgctttttagatgctaagcttgcacccgcatcgt

SEQ ID NO: 142 - DNA, 110 bp, synthetic construct
  source 1..110: mol_type = other DNA
cctgccacgctccgcaagcttccttctggtcctgcagcgattcttgatcggctatctcgcctatagtctcgacgtagtatgcaggcatgctaagcttgcacccgcatcgt

SEQ ID NO: 143 - DNA, 66 bp, synthetic construct
  source 1..66: mol_type = other DNA
cagcaccgtcaactgaattccgtggagccgtgggttatccgtgcgaccgtgatgcgatggagatgt

SEQ ID NO: 144 - DNA, 66 bp, synthetic construct
  source 1..66: mol_type = other DNA
cagcaccgtcaactgaatccgtgtggatccgtgcctgccgtgtccaccgtgatgcgatggagatgt

SEQ ID NO: 145 - DNA, 66 bp, synthetic construct
  source 1..66: mol_type = other DNA
cagcaccgtcaactgaatccgccgcgaccgtgtgttagccgtggagccgtgatgcgatggagatgt

SEQ ID NO: 146 - DNA, 66 bp, synthetic construct
  source 1..66: mol_type = other DNA
cagcaccgtcaactgaatccgcgggaaccgtgtctgaccgtgtgacccgtgatgcgatggagatgt

SEQ ID NO: 147 - DNA, 66 bp, synthetic construct
  source 1..66: mol_type = other DNA
cagcaccgtcaactgaatcgtgcaaagccgtatgatgtgcgtagccgtgtgatgcgatggagatgt

SEQ ID NO: 148 - DNA, 67 bp, synthetic construct
  source 1..67: mol_type = other DNA
cagcaccgtcaactgaatccgtgggcgcgcgcctttgctgctgcaacccgtgatgcgatggagatgt

SEQ ID NO: 149 - DNA, 66 bp, synthetic construct
  source 1..66: mol_type = other DNA
cagcaccgtcaactgaatccgtgtagagccgtgtatccgtgcggcaccgtgatgcgatggagatgt

SEQ ID NO: 150 - DNA, 61 bp, synthetic construct
  source 1..61: mol_type = other DNA
cagcaccgtcaactgaatcgtgggggagggtggggtgcgaaatgtgatgcgatggagatgt

SEQ ID NO: 151 - DNA, 66 bp, synthetic construct
  source 1..66: mol_type = other DNA
cagcaccgtcaactgaatcgtgcaaagccgtgtctccgtgcgtgccgtgtgatgcgatggagatgt

SEQ ID NO: 152 - DNA, 66 bp, synthetic construct
  source 1..66: mol_type = other DNA
cagcaccgtcaactgaatcgtgtgacccgtgtataccgtgggagccgtgtgatgcgatggagatgt

SEQ ID NO: 153 - DNA, 66 bp, synthetic construct
  source 1..66: mol_type = other DNA
cagcaccgtcaactgaatccgtgggagccgcgaaccaccgtgcgacccgtgatgcgatggagatgt

SEQ ID NO: 154 - DNA, 61 bp, synthetic construct
  source 1..61: mol_type = other DNA
cagcaccgtcaactgaatccgggcggcggcgggcccctgccgtgtgatgcgatggagatgt

SEQ ID NO: 155 - DNA, 66 bp, synthetic construct
  source 1..66: mol_type = other DNA
cagcaccgtcaactgaattctgggaaccgtgtgaaaccgtgtgaccgtgtgatgcgatggagatgt

SEQ ID NO: 156 - DNA, 66 bp, synthetic construct
  source 1..66: mol_type = other DNA
cagcaccgtcaactgaatgaggctctgaatccgtgtgaaaccgtgtgagtgatgcgatggagatgt

SEQ ID NO: 157 - DNA, 109 bp, synthetic construct
  source 1..109: mol_type = other DNA
ggaggctctcgggacgaccagcaccgtcaactgaattccgtggagccgtgggttatccgtgcgaccgtgatgcgatggagatgtgtcgtcccgatcacttgaatggtct

SEQ ID NO: 158 - DNA, 109 bp, synthetic construct
  source 1..109: mol_type = other DNA
ggaggctctcgggacgaccagcaccgtcaactgaatccgccgcgaccgtgtgttagccgtggagccgtgatgcgatggagatgtgtcgtcccgatcacttgaatggtct

SEQ ID NO: 159 - DNA, 109 bp, synthetic construct
  source 1..109: mol_type = other DNA
ggaggctctcgggacgaccagcaccgtcaactgaatccgcgggaaccgtgtctgaccgtgtgacccgtgatgcgatggagatgtgtcgtcccgatcacttgaatggtct

SEQ ID NO: 160 - DNA, 109 bp, synthetic construct
  source 1..109: mol_type = other DNA
ggaggctctcgggacgaccagcaccgtcaactgaatcgtgcaaagccgtatgatgtgcgtagccgtgtgatgcgatggagatgtgtcgtcccgatcacttgaatggtct

SEQ ID NO: 161 - DNA, 109 bp, synthetic construct
  source 1..109: mol_type = other DNA
ggaggctctcgggacgaccagcaccgtcaactgaatcgtgtgacccgtgtataccgtgggagccgtgtgatgcgatggagatgtgtcgtcccgatcacttgaatggtct

SEQ ID NO: 162 - DNA, 109 bp, synthetic construct
  source 1..109: mol_type = other DNA
ggaggctctcgggacgaccagcaccgtcaactgaattctgggaaccgtgtgaaaccgtgtgaccgtgtgatgcgatggagatgtgtcgtcccgatcacttgaatggtct

SEQ ID NO: 163 - protein, 244 aa, synthetic construct
EVQLVESGGGLVKPGGSLKLSCAASGLTFSGYAMSWFRQAPEKRLEWVATISSGGSYTYYLDSVKGRFTISRDNSKNTLYLQMSSLRSEDTAVYYCLASLITTDYFEYWGQGTLVTVSSASTKGPSVFPLAPSSKSTSGGTAALGCLVKDYFPEPVTVSWNSGALTSGVHTFPAVLQSSGLYSLSSVVTVPSSSLGTQTYICNVNHKPSNTKVDKKVEPKSCGGGSRLIEDICLPRWGCLWEDD

SEQ ID NO: 164 - protein, 214 aa, synthetic construct
DIVMTQSPSSLSASVGDRVTITCRASQDVGTAVAWYQQKPGQSPKLLIYWASTRYTGVPDRFSGSGSGTDFTLTISGLQSEDEADYFCQQYSNYPYTFGGGTKLEIKRTVAAPSVFIFPPSDEQLKSGTASVVCLLNNFYPREAKVQWKVDNALQSGNSQESVTEQDSKDSTYSLSSTLTLSKADYEKHKVYACEVTHQGLSSPVTKSFNRGEC